European Patent Application EP 4 393 505 A1, published July 3, 2024. Title: Vaccines for prevention of African swine fever comprising antigen proteins derived from African swine fever virus. Applicant: BioApplications Inc. The sequence listing filed with the application follows.

SEQUENCE LISTING (52 sequences)

SEQ ID NO: 1 - protein, 113 aa, synthetic construct
GEINKPICYQNDDKIFYCPKDWVGYNNVCYYFGNEEKNYNNASNYCKQLNSTLTNNNTILVNLTKTLNLTKTYNHESNYWVNYSLIKNESVLLRDSGYYKKQKHVSLLYICSK

SEQ ID NO: 2 - DNA, 339 bp, synthetic construct
  source 1..339: mol_type = other DNA
ggtgaaattaacaagccaatctgctaccaaaacgatgataagattttctactgtcctaaggattgggttggatacaacaacgtttgttactactttggcaacgaggaaaagaactataacaacgctagtaactactgcaagcagctgaactcgacattgacgaacaacaacactatcttggtgaacttaactaagaccctcaacctcacaaagacctacaaccatgagtctaactactgggtcaactactcactaattaagaacgagtctgtgcttcttagggacagcgggtactacaagaagcagaagcacgtttccttgctttacatatgctcaaag

SEQ ID NO: 3 - protein, 195 aa, synthetic construct
SNIVLSIDYWVSFNKTIILDSNITNDNNDINGVSWNFFNNSFNTLATCGKAGNFCECSNYSTSIYNITNNCSLTIFPHNDVFDTTYQVVWNQIINYTIKLLTPATPPNITYNCTNFLITCKKNNGTNTNIYLNINDTFVKYTNESILEYNWNNSNINNFTATCIINNTISTSNETTLINCTYLTLSSNYFYTFFK

SEQ ID NO: 4 - DNA, 585 bp, synthetic construct
  source 1..585: mol_type = other DNA
tctaacattgttcttagtattgattactgggtttcttttaataagacaatcatcctcgattctaacattactaacgacaataacgatattaatggagtgagttggaacttttttaacaacagctttaatactctagcaacatgcggtaaagctggcaatttttgcgagtgcagcaattactcaacaagtatatacaatatcaccaataattgctcccttacaatatttcctcataacgatgttttcgatactacatatcaggtcgtgtggaatcagattatcaactacacgatcaagcttttgacccctgctactcctcctaacataacctacaactgtactaattttctgataacgtgtaagaagaataacggtacaaacaccaacatttatctgaatataaatgacacgttcgtgaaatacactaacgaaagtatccttgagtataactggaataactccaatattaataacttcactgcaacttgtatcattaacaatactatttcaacttcgaacgaaacaaccttgataaattgtacgtacttaactctttcttccaattacttctataccttctttaag

SEQ ID NO: 5 - protein, 645 aa, synthetic construct
MASGGAFCLIANDGKADKIILAQDLLNSRISNIKNVNKSYGKPDPEPTLSQIEETHLVHFNAHFKPYVPVGFEYNKVRPHTGTPTLGNKLTFGIPQYGDFFHDMVGHHILGACHSSWQDAPIQGTSQMGAHGQLQTFPRNGYDWDNQTPLEGAVYTLVDPFGRPIVPGTKNAYRNLVYYCEYPGERLYENVRFDVNGNSLDEYSSDVTTLVRKFCIPGDKMTGYKHLVGQEVSVEGTSGPLLCNIHDLHKPHQSKPILTDENDTQRTCSHTNPKFLSQHFPENSHNIQTAGKQDITPITDATYLDIRRNVHYSCNGPQTPKYYQPPLALWIKLRFWFNENVNLAIPSVSIPFGERFITIKLASQKDLVNEFPGLFVRQSRFIAGRPSRRNIRFKPWFIPGVINEISLTNNELYINNLFVTPEIHNLFVKRVRFSLIRVHKTQVTHTNNNHHDEKLMSALKWPIEYMFIGLKPTWNISDQNPHQHRDWHKFGHVVNAIMQPTHHAEISFQDRDTALPDACSSISDISPVTYPITLPIIKNISVTAHGINLIDKFPSKFCSSYIPFHYGGNAIKTPDDPGAMMITFALKPREEYQPSGHINVSRAREFYISWDTDYVGSITTADLVVSASAINFLLLQNGSAVLRYS

SEQ ID NO: 6 - DNA, 1935 bp, synthetic construct
  source 1..1935: mol_type = other DNA
atggcttctggtggtgctttttgccttattgctaacgacgggaaagctgataagataatattagctcaggatctattgaactctaggatttcaaacatcaagaacgtcaacaagtcttacggtaagcctgatcctgaacctactcttagtcaaattgaagaaacccatcttgttcattttaatgcccattttaagccttatgttcctgttggttttgagtacaataaagtgagaccgcacactgggacgccaacccttggtaacaagctcacttttggtatccctcagtatggcgacttttttcatgatatggttggtcatcatattcttggcgcttgtcactcttcttggcaagatgctcctatacaaggtacctcgcaaatgggtgctcatggccagcttcagacgtttcctaggaatggttatgactgggataaccagacgcctcttgaaggcgctgtctatactctagttgatccttttggtagacctattgttcccggtactaagaatgcttatagaaaccttgtttactactgcgagtatcctggggaacgactttatgagaatgttaggttcgatgttaacggtaactctcttgatgagtactcttctgacgttactacgcttgttagaaagttttgtatccctggcgataagatgactggttataagcatcttgttggacaggaggtttctgttgaagggacgtccggtccacttctttgcaacattcatgaccttcacaagcctcatcaatctaagcctattcttactgatgagaatgacacacagagaacttgttctcatactaaccctaagttcctttctcaacacttccctgaaaacagccacaatattcagaccgctggaaagcaagacattacccctattactgatgcaacttatcttgatattaggcgcaatgttcattacagctgtaatggtccacaaactcccaagtattatcaaccgccgctggctctttggatcaagcttcgtttttggttcaatgagaacgttaatcttgcgatcccttctgtatctattccttttggtgagcgtttcattactattaagctagcttctcagaaggatctcgtaaatgagttccctggtctctttgtgcgccagtcccggtttattgctggtagacctagtcgtagaaacattagatttaaaccttggttcattcctggcgtgattaatgaaatttctcttactaacaacgaactttacattaacaatctttttgttactcctgaaattcacaaccttttcgtgaagagagtcagattttcactgattagagttcacaagacacaggttactcatactaataataatcatcacgacgaaaagcttatgtctgctctaaagtggcctatcgaatacatgtttatagggcttaagcccacttggaatatttctgatcagaatccacatcagcatagagattggcacaagttcggtcatgttgttaatgctattatgcaacctactcatcatgctgaaatctcttttcaagatagagatactgcccttccagatgcttgctcttctatttctgacattagccccgttacctacccgatcacccttcccatcatcaagaatatttctgttactgctcatggtattaatcttattgacaagtttccgtcgaagttctgttcttcttacattccctttcactacggtggtaatgctattaagactccggatgatcctggtgccatgatgattacttttgctcttaagcctcgggaggagtatcagccttctgggcatattaatgtttctagggctcgggaattttacatctcttgggacactgattatgttggttctattaccactgccgatcttgtcgtctctgcgtccgctatcaatttccttctccttcagaatggttctgccgtactccgttattct

SEQ ID NO: 7 - protein, 166 aa, synthetic construct
DSEFFQPVYPRHYGECLSPVTTPSFFSTHGGGGSSSRKKKAAAIEEEDIQFINPYQDQQWVEVTPQPGTSKPAGATTASVGKPVTGRPATNRPATNKPVTDNPVTDRLVMATGGPAAAPAAASAPAHPAEPYTTVTTQNTASQTMSAIENLRQRNTYTHKDLENSL

SEQ ID NO: 8 - DNA, 498 bp, synthetic construct
  source 1..498: mol_type = other DNA
gatagcgaatttttccagcctgtatatcctaggcattacggtgagtgcctctcaccagtgacaactcccagtttcttctctactcacggaggagggggttcatccagcagaaaaaaaaaggctgctgctatcgaggaagaagatattcaatttattaacccttatcaagatcaacagtgggtagaagttacaccacagcctggtacaagtaagcctgctggagcaacaaccgcttctgttggaaagcctgtcactgggagacctgctactaacagacctgctacaaataagccagtgactgataatccagttacagacaggcttgttatggctactggcggtccagctgctgctccagcagctgcttccgcacctgcacatccagcagagccttacactacagtgactactcaaaatactgcatcacagactatgtctgctatagagaatcttagacagagaaatacttatactcacaaagatttggaaaactctctt

SEQ ID NO: 9 - protein, 185 aa, synthetic construct
MKMEVIFKTDLRSSSQVVFHAGSLYNWFSVEIINSGRIVTTAIKTLLSTVKYDIVKSARIYAGQGYTEHQAQEEWNMILHVLFEEETESASSENIHEKNDNETNECTSSFETLFEQEPSSEVPKDSKLYMLAQKTVQHIEQYGKAPDFNKVIRAHNFIQTIYGTPLKEEEKEVVRLMVIKLLKKK

SEQ ID NO: 10 - DNA, 555 bp, synthetic construct
  source 1..555: mol_type = other DNA
atgaagatggaagtcatctttaagacagatcttaggtcatcttcacaagtagtattccatgcaggcagcctttataattggttctccgttgaaatcattaactctggacgtatagtgaccacggcaattaagacacttctgtcaactgttaagtatgacattgttaagagtgctagaatctacgcaggtcagggttatacagaacatcaagcccaagaggaatggaatatgattctccatgtgctctttgaggaggagactgagtctgctagttctgagaacattcacgagaagaacgataatgagacaaatgagtgtacctcgagttttgagactttgttcgaacaggagccttctagcgaggtgccaaaggactccaagttgtacatgctggcccagaagaccgttcagcacatcgagcagtacgggaaggctcctgattttaataaggtgattagggctcacaacttcatacaaactatttatggaactcctcttaaggaggaagagaaggaggttgttagattgatggtcataaagctattaaagaagaag

SEQ ID NO: 11 - protein, 159 aa, synthetic construct
PSNMKQFCKISVWLQQHDPDLLEIINNLCMLGNLSAAKYKHGVTFIYPKQAKIRDEIKKHAYSNDPSQAIKTLESLILPFYIPTPAEFTGEIGSYTGVKLEVEKTEANKVILKNGEAVLVPAADFKPFPDRRLAVWIMESGSMPLEGPPYKRKKEGGGN

SEQ ID NO: 12 - DNA, 477 bp, synthetic construct
  source 1..477: mol_type = other DNA
ccttcaaatatgaagcaattttgtaagatttctgtttggcttcaacagcatgatcccgacttgctcgaaataataaacaacctttgcatgttgggcaatttatcagcagctaagtacaaacatggagttaccttcatctatccgaagcaggctaagattcgtgacgagattaagaagcacgcatattctaatgatccgagtcaagctatcaagactttggagagcctgatactgccattctacattcctacacctgcagagtttacaggtgagattggatcttacacgggggttaaacttgaagtggagaagactgaagctaataaggtcatcctcaagaatggagaggccgtgcttgttcctgctgccgattttaagccattcccagatagaaggctagcggtatggattatggagtctggttccatgcctttggaaggtccaccctataagagaaagaaggagggcggtgggaac

SEQ ID NO: 13 - protein, 304 aa, synthetic construct
DPPVLKHISPYTPRTRIAIEVEKAFDDCMRQNWCSVNNPYLAKSVSLLSFLSLNHPTEFIKVLPLIDFDPLVTFYLLLEPYKTHGDDFLIPETILFGPTGWNGTDLYQSAMLEFKKFFTQITRQTFMDIADSATKEVDVPICYSDPETVHSYANHVRTEILHHNAVNKVTTPNLVVQAYNELEQTNTIRHYGPIFPESTINALRFWKKLWQDEQRFVIHGLHRTLMDQPTYETSEFAEIVRNLRFSRPGNNYINELNITSPAMYGDKHTTGDIAPNDRFAMLVAFINSTDFLYTAIPEEKVGGN

SEQ ID NO: 14 - DNA, 912 bp, synthetic construct
  source 1..912: mol_type = other DNA
gatccacctgtacttaagcacatctccccgtacacccctcgtactaggattgccatcgaagtagaaaaggcttttgacgattgtatgagacagaattggtgcagcgttaataacccgtatttggccaagtcggtttcccttcttagcttcttgagtctgaatcatccgactgagttcattaaagtcctcccccttattgatttcgaccctttggtgaccttttaccttttgctggagccttacaagactcacggcgatgatttcctcataccagaaactatactattcggtcctactggttggaacggaactgacctctatcaatctgcgatgcttgagttcaagaagtttttcacgcaaatcacccgacagacttttatggatatagcagattctgctacgaaggaggtcgatgtgcctatttgttactctgatcctgaaacagttcattcatatgcaaatcatgttagaaccgaaatccttcaccataacgctgttaataaggtgacaacccccaatcttgttgtgcaggcatataatgagctagagcaaactaacaccatcagacattacggccccattttcccagagagtaccattaatgctcttagattttggaagaagctttggcaagacgagcagcggtttgtaatccatggtttgcatcgtacattgatggatcagcctacctatgaaacttctgaatttgcagagattgttaggaaccttaggttttctcgccctgggaataactatataaacgaactgaatattacgtcacctgctatgtatggggataagcacactactggtgacattgccccaaatgatagattcgctatgcttgtcgcttttattaatagtaccgactttctttacacagctattcctgaagaaaaggtgggaggaaac

SEQ ID NO: 15 - protein, 185 aa, synthetic construct
SCMPVSTKCNDIWVDFSCTGPSISELQKKEPKAWAAILRSHTNQQTAEDDNIIGSICDKQGLCSKDEYAYSQYCACVNSGTLWAECAFAPCNGNKNAYKTTEQRNILTNKQCPSGLTICQNIAEYGGSGNISDLYQNFNCNSVINTEAAAKEAAAKYRLMSSSGGKHNDDKLPPPSLIFSNLNNF

SEQ ID NO: 16 - DNA, 555 bp, synthetic construct
  source 1..555: mol_type = other DNA
tcatgtatgcctgtttctactaagtgcaacgatatctgggttgatttttcatgtacaggaccttcaatttctgaattgcaaaagaaagagccaaaagcttgggctgctattcttagatcacatactaaccaacaaacagctgaagatgataacatcatcggatctatctgtgataagcaaggtttgtgctcaaaagatgagtatgcttactctcaatattgtgcttgcgttaattctggaactctttgggctgaatgtgcttttgctccttgcaacggtaacaagaacgcttacaagactacagagcaaagaaacattttgactaacaagcaatgtccatcaggacttacaatctgccaaaacatcgctgaatatggaggttcaggtaatatttctgatttgtaccaaaatttcaattgcaactctgttatcaacacagaagctgctgctaaggaggctgctgctaaatataggcttatgtcttcatctggaggtaaacataatgatgataaacttccacctccatcattgattttctctaatcttaataatttt

SEQ ID NO: 17 - protein, 316 aa, synthetic construct
VETQMDKLGFLLNHIGKQVTTKVLSNAHITQTMKEIILENHSVDGGAAKNVSKGKSSPKEKKHWTEFESWEQLSKSKRSFKEYWAERNEIVNTLLLNWDNVRGAIKKFLDDDREWCGRINMINGVPEIVEIIPSPYRAGENIYFGSEAMMPADIYSRVANKPAMFVFHTHPNLGSCCGGMPSICDISTTLRYLLMGWTAGHLIISSNQVGMLTVDKRIIVDLWANENPRWLMAQKILDIFMMLTSRRSLVNPWTLRDLKKILQDYGIEYIIFPSNDFFIYEDERLLMFSKKWTNFFTLHELLDDLETIETKASSTT

SEQ ID NO: 18 - DNA, 948 bp, synthetic construct
  source 1..948: mol_type = other DNA
gttgagactcaaatggataagcttggatttcttttgaaccatatcggaaagcaagttactacaaaggttctttctaacgctcatatcactcaaacaatgaaggaaatcattttggagaatcattctgttgatggaggtgctgctaagaatgtttcaaagggaaaatcttcaccaaaggaaaagaaacattggactgaattcgagtcttgggagcaactttctaagtcaaaaagatcattcaaggaatattgggctgaaaggaacgagatcgttaacacacttttgcttaactgggataatgttagaggtgctattaagaaatttttggatgatgatagagaatggtgtggaaggatcaacatgatcaacggtgttccagaaatcgttgagatcatcccatctccttacagagctggagaaaatatttactttggttctgaggctatgatgcctgctgatatttattcaagggttgctaacaagccagctatgtttgtttttcatacacatcctaaccttggatcatgttgcggaggtatgccatctatttgcgatatttcaactacattgaggtacttgcttatgggatggactgctggtcatttgatcatttcttcaaaccaagttggtatgcttacagttgataagagaatcatcgttgatttgtgggctaacgaaaatcctaggtggttgatggctcaaaagattcttgatattttcatgatgcttacttcaagaagatctcttgttaatccatggacattgagagatcttaagaaaattttgcaagattatggaattgagtacatcatcttcccttctaacgatttctttatctacgaagatgagaggttgcttatgttctcaaagaaatggactaatttctttacattgcatgaattgcttgatgatcttgaaactattgagacaaaggcttcttcaactaca

SEQ ID NO: 19 - protein, 27 aa, synthetic construct
MARSFGANSTVVLAIIFFGCLFALSSA

SEQ ID NO: 20 - DNA, 251 bp, synthetic construct
  source 1..251: mol_type = other DNA
atggctcgctcgtttggagctaacagtaccgttgtgttggcgatcatcttcttcggtgagtgattttccgatcttcttctccgatttagatctcctctacattgttgcttaatctcagaaccttttttcgttgttcctggatctgaatgtgtttgtttgcaatttcacgatcttaaaaggttagatctcgattggtattgacgattggaatctttacgatttcaggatgtttatttgcgttgtcctctgca

SEQ ID NO: 21 - protein, 34 aa, synthetic construct
MARSFGANSTVVLAIIFFGCLFALSSAIEEATKL

SEQ ID NO: 22 - DNA, 273 bp, synthetic construct
  source 1..273: mol_type = other DNA
atggctcgctcgtttggagctaacagtaccgttgtgttggcgatcatcttcttcggtgagtgattttccgatcttcttctccgatttagatctcctctacattgttgcttaatctcagaaccttttttcgttgttcctggatctgaatgtgtttgtttgcaatttcacgatcttaaaaggttagatctcgattggtattgacgattggaatctttacgatttcaggatgtttatttgcgttgtcctctgcaatagaagaggctacgaagttaa

SEQ ID NO: 23 - protein, 60 aa, synthetic construct
ANITVDYLYNKETKLFTAKLNVNENVECGNNTCTNNEVHNLTECKNASVSISHNSCTAPD

SEQ ID NO: 24 - DNA, 180 bp, synthetic construct
  source 1..180: mol_type = other DNA
gcaaacatcactgtggattacttatataacaaggaaactaaattatttacagcaaagctaaatgttaatgagaatgtggaatgtggaaacaatacttgcacaaacaatgaggtgcataaccttacagaatgtaaaaatgcgtctgtttccatatctcataattcatgtactgctcctgat

SEQ ID NO: 25 - protein, 6 aa, synthetic construct
HHHHHH

SEQ ID NO: 26 - DNA, 18 bp, synthetic construct
  source 1..18: mol_type = other DNA
caccaccatcaccaccat

SEQ ID NO: 27 - protein, 227 aa, synthetic construct
VGRPCPICPACEGPGPSAFIFPPKPKDTLMISRTPQVTCVVVDVSQENPEVQFSWYVDGVEVHTAQTRPKEAQFNSTYRVVSVLPIQHEDWLKGKEFECKVNNKDLPAPITRIISKAKGPSREPQVYTLSPSAEELSRSKVSITCLVTGFYPPDIDVEWKSNGQPEPEGNYRTTPPQQDVDGTYFLYSKLAVDKASWQRGDPFQCAVMHEALHNHYTQKSVSKTQGK

SEQ ID NO: 28 - DNA, 681 bp, synthetic construct
  source 1..681: mol_type = other DNA
gttggaagaccatgccctatatgtcctgcttgtgaaggtccaggtccctctgcttttatattcccaccaaagccgaaggataccttgatgatttcacgtacaccacaagttacttgtgttgttgtggatgtttcacaagaaaatcctgaggtacaattcagctggtatgttgatggggtagaagtgcacactgcacagactcgaccaaaggaggcccagtttaactcgacttatagagttgtttctgttctcccaatccaacacgaagattggctgaagggcaaggaatttgaatgcaaggttaacaataaagatctaccagcaccaattaccaggattatttctaaggcaaaaggaccctccagagagccccaagtttacacattgtctccttctgctgaggagcttagtagaagtaaagtgagcattacctgcttagtgacgggattctaccctccagacatcgacgtcgaatggaaatctaatggtcaacctgagccagaaggtaactataggactactccaccacaacaggacgtcgatggcacatactttctttattcaaaacttgctgtcgataaggcaagttggcaaagaggagatccatttcagtgtgctgtaatgcatgaggctttgcataatcattatacacagaaatcagtttctaaaacacaagggaaa

SEQ ID NO: 29 - protein, 4 aa, synthetic construct
HDEL

SEQ ID NO: 30 - DNA, 12 bp, synthetic construct
  source 1..12: mol_type = other DNA
cacgatgagctc

SEQ ID NO: 31 - protein, 356 aa, synthetic construct
HHHHHHGILGEINKPICYQNDDKIFYCPKDWVGYNNVCYYFGNEEKNYNNASNYCKQLNSTLTNNNTILVNLTKTLNLTKTYNHESNYWVNYSLIKNESVLLRDSGYYKKQKHVSLLYICSKPRAVGRPCPICPACEGPGPSAFIFPPKPKDTLMISRTPQVTCVVVDVSQENPEVQFSWYVDGVEVHTAQTRPKEAQFNSTYRVVSVLPIQHEDWLKGKEFECKVNNKDLPAPITRIISKAKGPSREPQVYTLSPSAEELSRSKVSITCLVTGFYPPDIDVEWKSNGQPEPEGNYRTTPPQQDVDGTYFLYSKLAVDKASWQRGDPFQCAVMHEALHNHYTQKSVSKTQGKHDEL

SEQ ID NO: 32 - DNA, 1355 bp, synthetic construct
  source 1..1355: mol_type = other DNA
tctagaattattacatcaaaacaaaaaatggctcgctcgtttggagctaacagtaccgttgtgttggcgatcatcttcttcggtgagtgattttccgatcttcttctccgatttagatctcctctacattgttgcttaatctcagaaccttttttcgttgttcctggatctgaatgtgtttgtttgcaatttcacgatcttaaaaggttagatctcgattggtattgacgattggaatctttacgatttcaggatgtttatttgcgttgtcctctgcacaccaccatcaccaccatgggatcctgggtgaaattaacaagccaatctgctaccaaaacgatgataagattttctactgtcctaaggattgggttggatacaacaacgtttgttactactttggcaacgaggaaaagaactataacaacgctagtaactactgcaagcagctgaactcgacattgacgaacaacaacactatcttggtgaacttaactaagaccctcaacctcacaaagacctacaaccatgagtctaactactgggtcaactactcactaattaagaacgagtctgtgcttcttagggacagcgggtactacaagaagcagaagcacgtttccttgctttacatatgctcaaagccccgggcagttggaagaccatgccctatatgtcctgcttgtgaaggtccaggtccctctgcttttatattcccaccaaagccgaaggataccttgatgatttcacgtacaccacaagttacttgtgttgttgtggatgtttcacaagaaaatcctgaggtacaattcagctggtatgttgatggggtagaagtgcacactgcacagactcgaccaaaggaggcccagtttaactcgacttatagagttgtttctgttctcccaatccaacacgaagattggctgaagggcaaggaatttgaatgcaaggttaacaataaagatctaccagcaccaattaccaggattatttctaaggcaaaaggaccctccagagagccccaagtttacacattgtctccttctgctgaggagcttagtagaagtaaagtgagcattacctgcttagtgacgggattctaccctccagacatcgacgtcgaatggaaatctaatggtcaacctgagccagaaggtaactataggactactccaccacaacaggacgtcgatggcacatactttctttattcaaaacttgctgtcgataaggcaagttggcaaagaggagatccatttcagtgtgctgtaatgcatgaggctttgcataatcattatacacagaaatcagtttctaaaacacaagggaaacacgatgagctctagctcgag

SEQ ID NO: 33 - protein, 491 aa, synthetic construct
ANITVDYLYNKETKLFTAKLNVNENVECGNNTCTNNEVHNLTECKNASVSISHNSCTAPDGSSNIVLSIDYWVSFNKTIILDSNITNDNNDINGVSWNFFNNSFNTLATCGKAGNFCECSNYSTSIYNITNNCSLTIFPHNDVFDTTYQVVWNQIINYTIKLLTPATPPNITYNCTNFLITCKKNNGTNTNIYLNINDTFVKYTNESILEYNWNNSNINNFTATCIINNTISTSNETTLINCTYLTLSSNYFYTFFKPRAVGRPCPICPACEGPGPSAFIFPPKPKDTLMISRTPQVTCVVVDVSQENPEVQFSWYVDGVEVHTAQTRPKEAQFNSTYRVVSVLPIQHEDWLKGKEFECKVNNKDLPAPITRIISKAKGPSREPQVYTLSPSAEELSRSKVSITCLVTGFYPPDIDVEWKSNGQPEPEGNYRTTPPQQDVDGTYFLYSKLAVDKASWQRGDPFQCAVMHEALHNHYTQKSVSKTQGKHDEL

SEQ ID NO: 34 - DNA, 1760 bp, synthetic construct
  source 1..1760: mol_type = other DNA
tctagaattattacatcaaaacaaaaaatggctcgctcgtttggagctaacagtaccgttgtgttggcgatcatcttcttcggtgagtgattttccgatcttcttctccgatttagatctcctctacattgttgcttaatctcagaaccttttttcgttgttcctggatctgaatgtgtttgtttgcaatttcacgatcttaaaaggttagatctcgattggtattgacgattggaatctttacgatttcaggatgtttatttgcgttgtcctctgcagcaaacatcactgtggattacttatataacaaggaaactaaattatttacagcaaagctaaatgttaatgagaatgtggaatgtggaaacaatacttgcacaaacaatgaggtgcataaccttacagaatgtaaaaatgcgtctgtttccatatctcataattcatgtactgctcctgatggatcctctaacattgttcttagtattgattactgggtttcttttaataagacaatcatcctcgattctaacattactaacgacaataacgatattaatggagtgagttggaacttttttaacaacagctttaatactctagcaacatgcggtaaagctggcaatttttgcgagtgcagcaattactcaacaagtatatacaatatcaccaataattgctcccttacaatatttcctcataacgatgttttcgatactacatatcaggtcgtgtggaatcagattatcaactacacgatcaagcttttgacccctgctactcctcctaacataacctacaactgtactaattttctgataacgtgtaagaagaataacggtacaaacaccaacatttatctgaatataaatgacacgttcgtgaaatacactaacgaaagtatccttgagtataactggaataactccaatattaataacttcactgcaacttgtatcattaacaatactatttcaacttcgaacgaaacaaccttgataaattgtacgtacttaactctttcttccaattacttctataccttctttaagccccgggcagttggaagaccatgccctatatgtcctgcttgtgaaggtccaggtccctctgcttttatattcccaccaaagccgaaggataccttgatgatttcacgtacaccacaagttacttgtgttgttgtggatgtttcacaagaaaatcctgaggtacaattcagctggtatgttgatggggtagaagtgcacactgcacagactcgaccaaaggaggcccagtttaactcgacttatagagttgtttctgttctcccaatccaacacgaagattggctgaagggcaaggaatttgaatgcaaggttaacaataaagatctaccagcaccaattaccaggattatttctaaggcaaaaggaccctccagagagccccaagtttacacattgtctccttctgctgaggagcttagtagaagtaaagtgagcattacctgcttagtgacgggattctaccctccagacatcgacgtcgaatggaaatctaatggtcaacctgagccagaaggtaactataggactactccaccacaacaggacgtcgatggcacatactttctttattcaaaacttgctgtcgataaggcaagttggcaaagaggagatccatttcagtgtgctgtaatgcatgaggctttgcataatcattatacacagaaatcagtttctaaaacacaagggaaacacgatgagctctagctcgag

SEQ ID NO: 35 - protein, 889 aa, synthetic construct
IEEATKLRILMASGGAFCLIANDGKADKIILAQDLLNSRISNIKNVNKSYGKPDPEPTLSQIEETHLVHFNAHFKPYVPVGFEYNKVRPHTGTPTLGNKLTFGIPQYGDFFHDMVGHHILGACHSSWQDAPIQGTSQMGAHGQLQTFPRNGYDWDNQTPLEGAVYTLVDPFGRPIVPGTKNAYRNLVYYCEYPGERLYENVRFDVNGNSLDEYSSDVTTLVRKFCIPGDKMTGYKHLVGQEVSVEGTSGPLLCNIHDLHKPHQSKPILTDENDTQRTCSHTNPKFLSQHFPENSHNIQTAGKQDITPITDATYLDIRRNVHYSCNGPQTPKYYQPPLALWIKLRFWFNENVNLAIPSVSIPFGERFITIKLASQKDLVNEFPGLFVRQSRFIAGRPSRRNIRFKPWFIPGVINEISLTNNELYINNLFVTPEIHNLFVKRVRFSLIRVHKTQVTHTNNNHHDEKLMSALKWPIEYMFIGLKPTWNISDQNPHQHRDWHKFGHVVNAIMQPTHHAEISFQDRDTALPDACSSISDISPVTYPITLPIIKNISVTAHGINLIDKFPSKFCSSYIPFHYGGNAIKTPDDPGAMMITFALKPREEYQPSGHINVSRAREFYISWDTDYVGSITTADLVVSASAINFLLLQNGSAVLRYSTRAVGRPCPICPACEGPGPSAFIFPPKPKDTLMISRTPQVTCVVVDVSQENPEVQFSWYVDGVEVHTAQTRPKEAQFNSTYRVVSVLPIQHEDWLKGKEFECKVNNKDLPAPITRIISKAKGPSREPQVYTLSPSAEELSRSKVSITCLVTGFYPPDIDVEWKSNGQPEPEGNYRTTPPQQDVDGTYFLYSKLAVDKASWQRGDPFQCAVMHEALHNHYTQKSVSKTQGKHDEL

SEQ ID NO: 36 - DNA, 2954 bp, synthetic construct
  source 1..2954: mol_type = other DNA
tctagaattattacatcaaaacaaaaaatggctcgctcgtttggagctaacagtaccgttgtgttggcgatcatcttcttcggtgagtgattttccgatcttcttctccgatttagatctcctctacattgttgcttaatctcagaaccttttttcgttgttcctggatctgaatgtgtttgtttgcaatttcacgatcttaaaaggttagatctcgattggtattgacgattggaatctttacgatttcaggatgtttatttgcgttgtcctctgcaatagaagaggctacgaagttaaggatccttatggcttctggtggtgctttttgccttattgctaacgacgggaaagctgataagataatattagctcaggatctattgaactctaggatttcaaacatcaagaacgtcaacaagtcttacggtaagcctgatcctgaacctactcttagtcaaattgaagaaacccatcttgttcattttaatgcccattttaagccttatgttcctgttggttttgagtacaataaagtgagaccgcacactgggacgccaacccttggtaacaagctcacttttggtatccctcagtatggcgacttttttcatgatatggttggtcatcatattcttggcgcttgtcactcttcttggcaagatgctcctatacaaggtacctcgcaaatgggtgctcatggccagcttcagacgtttcctaggaatggttatgactgggataaccagacgcctcttgaaggcgctgtctatactctagttgatccttttggtagacctattgttcccggtactaagaatgcttatagaaaccttgtttactactgcgagtatcctggggaacgactttatgagaatgttaggttcgatgttaacggtaactctcttgatgagtactcttctgacgttactacgcttgttagaaagttttgtatccctggcgataagatgactggttataagcatcttgttggacaggaggtttctgttgaagggacgtccggtccacttctttgcaacattcatgaccttcacaagcctcatcaatctaagcctattcttactgatgagaatgacacacagagaacttgttctcatactaaccctaagttcctttctcaacacttccctgaaaacagccacaatattcagaccgctggaaagcaagacattacccctattactgatgcaacttatcttgatattaggcgcaatgttcattacagctgtaatggtccacaaactcccaagtattatcaaccgccgctggctctttggatcaagcttcgtttttggttcaatgagaacgttaatcttgcgatcccttctgtatctattccttttggtgagcgtttcattactattaagctagcttctcagaaggatctcgtaaatgagttccctggtctctttgtgcgccagtcccggtttattgctggtagacctagtcgtagaaacattagatttaaaccttggttcattcctggcgtgattaatgaaatttctcttactaacaacgaactttacattaacaatctttttgttactcctgaaattcacaaccttttcgtgaagagagtcagattttcactgattagagttcacaagacacaggttactcatactaataataatcatcacgacgaaaagcttatgtctgctctaaagtggcctatcgaatacatgtttatagggcttaagcccacttggaatatttctgatcagaatccacatcagcatagagattggcacaagttcggtcatgttgttaatgctattatgcaacctactcatcatgctgaaatctcttttcaagatagagatactgcccttccagatgcttgctcttctatttctgacattagccccgttacctacccgatcacccttcccatcatcaagaatatttctgttactgctcatggtattaatcttattgacaagtttccgtcgaagttctgttcttcttacattccctttcactacggtggtaatgctattaagactccggatgatcctggtgccatgatgattacttttgctcttaagcctcgggaggagtatcagccttctgggcatattaatgtttctagggctcgggaattttacatctcttgggacactgattatgttggttctattaccactgccgatcttgtcgtctctgcgtccgctatcaatttccttctccttcagaatggttctgccgtactccgttattctacccgggcagttggaagaccatgccctatatgtcctgcttgtgaaggtccaggtccctctgcttttatattcccaccaaagccgaaggataccttgatgatttcacgtacaccacaagttacttgtgttgttgtggatgtttcacaagaaaatcctgaggtacaattcagctggtatgttgatggggtagaagtgcacactgcacagactcgaccaaaggaggcccagtttaactcgacttatagagttgtttctgttctcccaatccaacacgaagattggctgaagggcaaggaatttgaatgcaaggttaacaataaagatctaccagcaccaattaccaggattatttctaaggcaaaaggaccctccagagagccccaagtttacacattgtctccttctgctgaggagcttagtagaagtaaagtgagcattacctgcttagtgacgggattctaccctccagacatcgacgtcgaatggaaatctaatggtcaacctgagccagaaggtaactataggactactccaccacaacaggacgtcgatggcacatactttctttattcaaaacttgctgtcgataaggcaagttggcaaagaggagatccatttcagtgtgctgtaatgcatgaggctttgcataatcattatacacagaaatcagtttctaaaacacaagggaaacacgatgagctctagctcgag

SEQ ID NO: 37 - protein, 402 aa, synthetic construct
GSDSEFFQPVYPRHYGECLSPVTTPSFFSTHGGGGSSSRKKKAAAIEEEDIQFINPYQDQQWVEVTPQPGTSKPAGATTASVGKPVTGRPATNRPATNKPVTDNPVTDRLVMATGGPAAAPAAASAPAHPAEPYTTVTTQNTASQTMSAIENLRQRNTYTHKDLENSLSRAVGRPCPICPACEGPGPSAFIFPPKPKDTLMISRTPQVTCVVVDVSQENPEVQFSWYVDGVEVHTAQTRPKEAQFNSTYRVVSVLPIQHEDWLKGKEFECKVNNKDLPAPITRIISKAKGPSREPQVYTLSPSAEELSRSKVSITCLVTGFYPPDIDVEWKSNGQPEPEGNYRTTPPQQDVDGTYFLYSKLAVDKASWQRGDPFQCAVMHEALHNHYTQKSVSKTQGKHDEL

SEQ ID NO: 38 - DNA, 1493 bp, synthetic construct
  source 1..1493: mol_type = other DNA
tctagaattattacatcaaaacaaaaaatggctcgctcgtttggagctaacagtaccgttgtgttggcgatcatcttcttcggtgagtgattttccgatcttcttctccgatttagatctcctctacattgttgcttaatctcagaaccttttttcgttgttcctggatctgaatgtgtttgtttgcaatttcacgatcttaaaaggttagatctcgattggtattgacgattggaatctttacgatttcaggatgtttatttgcgttgtcctctgcaggatccgatagcgaatttttccagcctgtatatcctaggcattacggtgagtgcctctcaccagtgacaactcccagtttcttctctactcacggaggagggggttcatccagcagaaaaaaaaaggctgctgctatcgaggaagaagatattcaatttattaacccttatcaagatcaacagtgggtagaagttacaccacagcctggtacaagtaagcctgctggagcaacaaccgcttctgttggaaagcctgtcactgggagacctgctactaacagacctgctacaaataagccagtgactgataatccagttacagacaggcttgttatggctactggcggtccagctgctgctccagcagctgcttccgcacctgcacatccagcagagccttacactacagtgactactcaaaatactgcatcacagactatgtctgctatagagaatcttagacagagaaatacttatactcacaaagatttggaaaactctctttcccgggcagttggaagaccatgccctatatgtcctgcttgtgaaggtccaggtccctctgcttttatattcccaccaaagccgaaggataccttgatgatttcacgtacaccacaagttacttgtgttgttgtggatgtttcacaagaaaatcctgaggtacaattcagctggtatgttgatggggtagaagtgcacactgcacagactcgaccaaaggaggcccagtttaactcgacttatagagttgtttctgttctcccaatccaacacgaagattggctgaagggcaaggaatttgaatgcaaggttaacaataaagatctaccagcaccaattaccaggattatttctaaggcaaaaggaccctccagagagccccaagtttacacattgtctccttctgctgaggagcttagtagaagtaaagtgagcattacctgcttagtgacgggattctaccctccagacatcgacgtcgaatggaaatctaatggtcaacctgagccagaaggtaactataggactactccaccacaacaggacgtcgatggcacatactttctttattcaaaacttgctgtcgataaggcaagttggcaaagaggagatccatttcagtgtgctgtaatgcatgaggctttgcataatcattatacacagaaatcagtttctaaaacacaagggaaacatgatgagctctagctcgag

SEQ ID NO: 39 - protein, 199 aa, synthetic construct
GSMKMEVIFKTDLRSSSQVVFHAGSLYNWFSVEIINSGRIVTTAIKTLLSTVKYDIVKSARIYAGQGYTEHQAQEEWNMILHVLFEEETESASSENIHEKNDNETNECTSSFETLFEQEPSSEVPKDSKLYMLAQKTVQHIEQYGKAPDFNKVIRAHNFIQTIYGTPLKEEEKEVVRLMVIKLLKKKSRGHHHHHHDEL

SEQ ID NO: 40 - DNA, 884 bp, synthetic construct
  source 1..884: mol_type = other DNA
tctagaattattacatcaaaacaaaaaatggctcgctcgtttggagctaacagtaccgttgtgttggcgatcatcttcttcggtgagtgattttccgatcttcttctccgatttagatctcctctacattgttgcttaatctcagaaccttttttcgttgttcctggatctgaatgtgtttgtttgcaatttcacgatcttaaaaggttagatctcgattggtattgacgattggaatctttacgatttcaggatgtttatttgcgttgtcctctgcaggatccatgaagatggaagtcatctttaagacagatcttaggtcatcttcacaagtagtattccatgcaggcagcctttataattggttctccgttgaaatcattaactctggacgtatagtgaccacggcaattaagacacttctgtcaactgttaagtatgacattgttaagagtgctagaatctacgcaggtcagggttatacagaacatcaagcccaagaggaatggaatatgattctccatgtgctctttgaggaggagactgagtctgctagttctgagaacattcacgagaagaacgataatgagacaaatgagtgtacctcgagttttgagactttgttcgaacaggagccttctagcgaggtgccaaaggactccaagttgtacatgctggcccagaagaccgttcagcacatcgagcagtacgggaaggctcctgattttaataaggtgattagggctcacaacttcatacaaactatttatggaactcctcttaaggaggaagagaaggaggttgttagattgatggtcataaagctattaaagaagaagtcccggggtcaccaccatcaccaccatgatgagctctagctcgag

SEQ ID NO: 41 - DNA, 24 bp, synthetic construct
  source 1..24: mol_type = other DNA
gcgatgatgattacctttgctttg

SEQ ID NO: 42 - DNA, 24 bp, synthetic construct
  source 1..24: mol_type = other DNA
cgatgatgattaccttcgctttga

SEQ ID NO: 43 - DNA, 21 bp, synthetic construct
  source 1..21: mol_type = other DNA
cgataccacaagatcagccgt

SEQ ID NO: 44 - DNA, 22 bp, synthetic construct
  source 1..22: mol_type = other DNA
ctgataccacaagatcagccgt

SEQ ID NO: 45 - DNA, 20 bp, synthetic construct
  source 1..20: mol_type = other DNA
gataccacaagatcggccgt

SEQ ID NO: 46 - DNA, 22 bp, synthetic construct
  source 1..22: mol_type = other DNA
cacgggaggaataccaacccag

SEQ ID NO: 47 - DNA, 1472 bp, synthetic construct
  source 1..1472: mol_type = other DNA
tctagaattattacatcaaaacaaaaaatggctcgctcgtttggagctaacagtaccgttgtgttggcgatcatcttcttcggtgagtgattttccgatcttcttctccgatttagatctcctctacattgttgcttaatctcagaaccttttttcgttgttcctggatctgaatgtgtttgtttgcaatttcacgatcttaaaaggttagatctcgattggtattgacgattggaatctttacgatttcaggatgtttatttgcgttgtcctctgcaggatccccttcaaatatgaagcaattttgtaagatttctgtttggcttcaacagcatgatcccgacttgctcgaaataataaacaacctttgcatgttgggcaatttatcagcagctaagtacaaacatggagttaccttcatctatccgaagcaggctaagattcgtgacgagattaagaagcacgcatattctaatgatccgagtcaagctatcaagactttggagagcctgatactgccattctacattcctacacctgcagagtttacaggtgagattggatcttacacgggggttaaacttgaagtggagaagactgaagctaataaggtcatcctcaagaatggagaggccgtgcttgttcctgctgccgattttaagccattcccagatagaaggctagcggtatggattatggagtctggttccatgcctttggaaggtccaccctataagagaaagaaggagggcggtgggaacccccgggcagttggaagaccatgccctatatgtcctgcttgtgaaggtccaggtccctctgcttttatattcccaccaaagccgaaggataccttgatgatttcacgtacaccacaagttacttgtgttgttgtggatgtttcacaagaaaatcctgaggtacaattcagctggtatgttgatggggtagaagtgcacactgcacagactcgaccaaaggaggcccagtttaactcgacttatagagttgtttctgttctcccaatccaacacgaagattggctgaagggcaaggaatttgaatgcaaggttaacaataaagatctaccagcaccaattaccaggattatttctaaggcaaaaggaccctccagagagccccaagtttacacattgtctccttctgctgaggagcttagtagaagtaaagtgagcattacctgcttagtgacgggattctaccctccagacatcgacgtcgaatggaaatctaatggtcaacctgagccagaaggtaactataggactactccaccacaacaggacgtcgatggcacatactttctttattcaaaacttgctgtcgataaggcaagttggcaaagaggagatccatttcagtgtgctgtaatgcatgaggctttgcataatcattatacacagaaatcagtttctaaaacacaagggaaacacgatgagctctagctcgag

SEQ ID NO: 48 - DNA, 1907 bp, synthetic construct
  source 1..1907: mol_type = other DNA
tctagaattattacatcaaaacaaaaaatggctcgctcgtttggagctaacagtaccgttgtgttggcgatcatcttcttcggtgagtgattttccgatcttcttctccgatttagatctcctctacattgttgcttaatctcagaaccttttttcgttgttcctggatctgaatgtgtttgtttgcaatttcacgatcttaaaaggttagatctcgattggtattgacgattggaatctttacgatttcaggatgtttatttgcgttgtcctctgcaggatccgatccacctgtacttaagcacatctccccgtacacccctcgtactaggattgccatcgaagtagaaaaggcttttgacgattgtatgagacagaattggtgcagcgttaataacccgtatttggccaagtcggtttcccttcttagcttcttgagtctgaatcatccgactgagttcattaaagtcctcccccttattgatttcgaccctttggtgaccttttaccttttgctggagccttacaagactcacggcgatgatttcctcataccagaaactatactattcggtcctactggttggaacggaactgacctctatcaatctgcgatgcttgagttcaagaagtttttcacgcaaatcacccgacagacttttatggatatagcagattctgctacgaaggaggtcgatgtgcctatttgttactctgatcctgaaacagttcattcatatgcaaatcatgttagaaccgaaatccttcaccataacgctgttaataaggtgacaacccccaatcttgttgtgcaggcatataatgagctagagcaaactaacaccatcagacattacggccccattttcccagagagtaccattaatgctcttagattttggaagaagctttggcaagacgagcagcggtttgtaatccatggtttgcatcgtacattgatggatcagcctacctatgaaacttctgaatttgcagagattgttaggaaccttaggttttctcgccctgggaataactatataaacgaactgaatattacgtcacctgctatgtatggggataagcacactactggtgacattgccccaaatgatagattcgctatgcttgtcgcttttattaatagtaccgactttctttacacagctattcctgaagaaaaggtgggaggaaacccccgggcagttggaagaccatgccctatatgtcctgcttgtgaaggtccaggtccctctgcttttatattcccaccaaagccgaaggataccttgatgatttcacgtacaccacaagttacttgtgttgttgtggatgtttcacaagaaaatcctgaggtacaattcagctggtatgttgatggggtagaagtgcacactgcacagactcgaccaaaggaggcccagtttaactcgacttatagagttgtttctgttctcccaatccaacacgaagattggctgaagggcaaggaatttgaatgcaaggttaacaataaagatctaccagcaccaattaccaggattatttctaaggcaaaaggaccctccagagagccccaagtttacacattgtctccttctgctgaggagcttagtagaagtaaagtgagcattacctgcttagtgacgggattctaccctccagacatcgacgtcgaatggaaatctaatggtcaacctgagccagaaggtaactataggactactccaccacaacaggacgtcgatggcacatactttctttattcaaaacttgctgtcgataaggcaagttggcaaagaggagatccatttcagtgtgctgtaatgcatgaggctttgcataatcattatacacagaaatcagtttctaaaacacaagggaaacacgatgagctctagctcgag

SEQ ID NO: 49 - DNA, 1550 bp, synthetic construct
  source 1..1550: mol_type = other DNA
tctagaattattacatcaaaacaaaaaatggctcgctcgtttggagctaacagtaccgttgtgttggcgatcatcttcttcggtgagtgattttccgatcttcttctccgatttagatctcctctacattgttgcttaatctcagaaccttttttcgttgttcctggatctgaatgtgtttgtttgcaatttcacgatcttaaaaggttagatctcgattggtattgacgattggaatctttacgatttcaggatgtttatttgcgttgtcctctgcaggatcctcatgtatgcctgtttctactaagtgcaacgatatctgggttgatttttcatgtacaggaccttcaatttctgaattgcaaaagaaagagccaaaagcttgggctgctattcttagatcacatactaaccaacaaacagctgaagatgataacatcatcggatctatctgtgataagcaaggtttgtgctcaaaagatgagtatgcttactctcaatattgtgcttgcgttaattctggaactctttgggctgaatgtgcttttgctccttgcaacggtaacaagaacgcttacaagactacagagcaaagaaacattttgactaacaagcaatgtccatcaggacttacaatctgccaaaacatcgctgaatatggaggttcaggtaatatttctgatttgtaccaaaatttcaattgcaactctgttatcaacacagaagctgctgctaaggaggctgctgctaaatataggcttatgtcttcatctggaggtaaacataatgatgataaacttccacctccatcattgattttctctaatcttaataattttccccgggcagttggaagaccatgccctatatgtcctgcttgtgaaggtccaggtccctctgcttttatattcccaccaaagccgaaggataccttgatgatttcacgtacaccacaagttacttgtgttgttgtggatgtttcacaagaaaatcctgaggtacaattcagctggtatgttgatggggtagaagtgcacactgcacagactcgaccaaaggaggcccagtttaactcgacttatagagttgtttctgttctcccaatccaacacgaagattggctgaagggcaaggaatttgaatgcaaggttaacaataaagatctaccagcaccaattaccaggattatttctaaggcaaaaggaccctccagagagccccaagtttacacattgtctccttctgctgaggagcttagtagaagtaaagtgagcattacctgcttagtgacgggattctaccctccagacatcgacgtcgaatggaaatctaatggtcaacctgagccagaaggtaactataggactactccaccacaacaggacgtcgatggcacatactttctttattcaaaacttgctgtcgataaggcaagttggcaaagaggagatccatttcagtgtgctgtaatgcatgaggctttgcataatcattatacacagaaatcagtttctaaaacacaagggaaacatgatgagctctagctcgag

SEQ ID NO: 50 - DNA, 1943 bp, synthetic construct
  source 1..1943: mol_type = other DNA
tctagaattattacatcaaaacaaaaaatggctcgctcgtttggagctaacagtaccgttgtgttggcgatcatcttcttcggtgagtgattttccgatcttcttctccgatttagatctcctctacattgttgcttaatctcagaaccttttttcgttgttcctggatctgaatgtgtttgtttgcaatttcacgatcttaaaaggttagatctcgattggtattgacgattggaatctttacgatttcaggatgtttatttgcgttgtcctctgcaggatccgttgagactcaaatggataagcttggatttcttttgaaccatatcggaaagcaagttactacaaaggttctttctaacgctcatatcactcaaacaatgaaggaaatcattttggagaatcattctgttgatggaggtgctgctaagaatgtttcaaagggaaaatcttcaccaaaggaaaagaaacattggactgaattcgagtcttgggagcaactttctaagtcaaaaagatcattcaaggaatattgggctgaaaggaacgagatcgttaacacacttttgcttaactgggataatgttagaggtgctattaagaaatttttggatgatgatagagaatggtgtggaaggatcaacatgatcaacggtgttccagaaatcgttgagatcatcccatctccttacagagctggagaaaatatttactttggttctgaggctatgatgcctgctgatatttattcaagggttgctaacaagccagctatgtttgtttttcatacacatcctaaccttggatcatgttgcggaggtatgccatctatttgcgatatttcaactacattgaggtacttgcttatgggatggactgctggtcatttgatcatttcttcaaaccaagttggtatgcttacagttgataagagaatcatcgttgatttgtgggctaacgaaaatcctaggtggttgatggctcaaaagattcttgatattttcatgatgcttacttcaagaagatctcttgttaatccatggacattgagagatcttaagaaaattttgcaagattatggaattgagtacatcatcttcccttctaacgatttctttatctacgaagatgagaggttgcttatgttctcaaagaaatggactaatttctttacattgcatgaattgcttgatgatcttgaaactattgagacaaaggcttcttcaactacaccccgggcagttggaagaccatgccctatatgtcctgcttgtgaaggtccaggtccctctgcttttatattcccaccaaagccgaaggataccttgatgatttcacgtacaccacaagttacttgtgttgttgtggatgtttcacaagaaaatcctgaggtacaattcagctggtatgttgatggggtagaagtgcacactgcacagactcgaccaaaggaggcccagtttaactcgacttatagagttgtttctgttctcccaatccaacacgaagattggctgaagggcaaggaatttgaatgcaaggttaacaataaagatctaccagcaccaattaccaggattatttctaaggcaaaaggaccctccagagagccccaagtttacacattgtctccttctgctgaggagcttagtagaagtaaagtgagcattacctgcttagtgacgggattctaccctccagacatcgacgtcgaatggaaatctaatggtcaacctgagccagaaggtaactataggactactccaccacaacaggacgtcgatggcacatactttctttattcaaaacttgctgtcgataaggcaagttggcaaagaggagatccatttcagtgtgctgtaatgcatgaggctttgcataatcattatacacagaaatcagtttctaaaacacaagggaaacatgatgagctctagctcgag

SEQ ID NO: 51 - protein, 5 aa, synthetic construct
GGGGS

SEQ ID NO: 52 - protein, 4 aa, synthetic construct
KDEL